European Patent Specification EP 3 789 397 B1, published December 6, 2023. Title: NOVEL SPECIFIC-BINDING POLYPEPTIDES AND USES THEREOF. Applicant: Pieris Pharmaceuticals GmbH. The sequence listing filed with the application follows.

SEQUENCE LISTING (68 sequences)

SEQ ID NO: 1 - protein, 151 aa, artificial
  lipocalin mutein
ASDEEIQDVSGTWYLKAMTVDFWCSGIHEESVTPMTLTTLEGGNLEAKVTMDIEGFLQEFKAVLEKTDEPGKYTADGGKHVAYIIRSRVKDHYIFYSEGDCPGPVPGVWLVGRDPKNNLEALEDFEKAAGARGLSTESILIPRQSETSSPG

SEQ ID NO: 2 - protein, 178 aa, artificial
  lipocalin mutein
QDSTSDLIPAPPLSKVPLQQNFQDNQFHGKWYVVGEAGNLLLREDKDPRKMTATIYELKEDKSYDVTRVEFGAKTYKYQIGTFVPGSQPGEFTLGGIESMPGMTSFLVRVVSTNYNQHAIVFFKYVYQNREYFEITLYGRTKELTSELKENFIRFSKSLGLPENHIVFPVPIDQAIDG

SEQ ID NO: 3 - protein, 351 aa, artificial
  fusion protein
ASDEEIQDVSGTWYLKAMTVDFWCSGIHEESVTPMTLTTLEGGNLEAKVTMDIEGFLQEFKAVLEKTDEPGKYTADGGKHVAYIIRSRVKDHYIFYSEGDCPGPVPGVWLVGRDPKNNLEALEDFEKAAGARGLSTESILIPRQSETSSPGSDGGGGSGGGGSQDSTSDLIPAPPLSKVPLQQNFQDNQFHGKWYVVGEAGNLLLREDKDPRKMTATIYELKEDKSYDVTRVEFGAKTYKYQIGTFVPGSQPGEFTLGGIESMPGMTSFLVRVVSTNYNQHAIVFFKYVYQNREYFEITLYGRTKELTSELKENFIRFSKSLGLPENHIVFPVPIDQAIDGSAWSHPQFEK

SEQ ID NO: 4 - protein, 349 aa, artificial
  fusion protein
QDSTSDLIPAPPLSKVPLQQNFQDNQFHGKWYVVGEAGNLLLREDKDPRKMTATIYELKEDKSYDVTRVEFGAKTYKYQIGTFVPGSQPGEFTLGGIESMPGMTSFLVRVVSTNYNQHAIVFFKYVYQNREYFEITLYGRTKELTSELKENFIRFSKSLGLPENHIVFPVPIDQAIDGGGGGSGGGGSASDEEIQDVSGTWYLKAMTVDFWCSGIHEESVTPMTLTTLEGGNLEAKVTMDIEGFLQEFKAVLEKTDEPGKYTADGGKHVAYIIRSRVKDHYIFYSEGDCPGPVPGVWLVGRDPKNNLEALEDFEKAAGARGLSTESILIPRQSETSSPGSAWSHPQFEK

SEQ ID NO: 5 - protein, 406 aa, artificial
  fusion protein
ASDEEIQDVSGTWYLKAMTVDFWCSGIHEESVTPMTLTTLEGGNLEAKVTMDIEGFLQEFKAVLEKTDEPGKYTADGGKHVAYIIRSRVKDHYIFYSEGDCPGPVPGVWLVGRDPKNNLEALEDFEKAAGARGLSTESILIPRQSETSSPGSDGGGGSGGGGSQDSTSDLIPAPPLSKVPLQQNFQDNQFHGKWYVVGEAGNLLLREDKDPRKMTATIYELKEDKSYDVTRVEFGAKTYKYQIGTFVPGSQPGEFTLGGIESMPGMTSFLVRVVSTNYNQHAIVFFKYVYQNREYFEITLYGRTKELTSELKENFIRFSKSLGLPENHIVFPVPIDQAIDGSAGAVDANSLAEAKVLANRELDKYGVSDYYKNLINNAKTVEGVKALIDEILAALPSAWSHPQFEK

SEQ ID NO: 6 - protein, 556 aa, artificial
  fusion protein
ASDEEIQDVSGTWYLKAMTVDFWCSGIHEESVTPMTLTTLEGGNLEAKVTMDIEGFLQEFKAVLEKTDEPGKYTADGGKHVAYIIRSRVKDHYIFYSEGDCPGPVPGVWLVGRDPKNNLEALEDFEKAAGARGLSTESILIPRQSETSSPGSDGGGGSGGGGSASDEEIQDVSGTWYLKAMTVDFWCSGIHEESVTPMTLTTLEGGNLEAKVTMDIEGFLQEFKAVLEKTDEPGKYTADGGKHVAYIIRSRVKDHYIFYSEGDCPGPVPGVWLVGRDPKNNLEALEDFEKAAGARGLSTESILIPRQSETSSPGSDGGGGSGGGGSQDSTSDLIPAPPLSKVPLQQNFQDNQFHGKWYVVGEAGNLLLREDKDPRKMTATIYELKEDKSYDVTRVEFGAKTYKYQIGTFVPGSQPGEFTLGGIESMPGMTSFLVRVVSTNYNQHAIVFFKYVYQNREYFEITLYGRTKELTSELKENFIRFSKSLGLPENHIVFPVPIDQAIDGSGGGGSLAEAKEAANAELDSYGVSDFYKRLIDKAKTVEGVEALKDAILAALP

SEQ ID NO: 7 - protein, 240 aa, artificial
  fusion protein
QDSTSDLIPAPPLSKVPLQQNFQDNQFHGKWYVVGEAGNLLLREDKDPRKMTATIYELKEDKSYDVTRVEFGAKTYKYQIGTFVPGSQPGEFTLGGIESMPGMTSFLVRVVSTNYNQHAIVFFKYVYQNREYFEITLYGRTKELTSELKENFIRFSKSLGLPENHIVFPVPIDQAIDGSGGGGSLAEAKEAANAELDSYGVSDFYKRLIDKAKTVEGVEALKDAILAALPSAWSHPQFEK

SEQ ID NO: 8 - protein, 215 aa, artificial
  fusion protein
ASDEEIQDVSGTWYLKAMTVDFWCSGIHEESVTPMTLTTLEGGNLEAKVTMDIEGFLQEFKAVLEKTDEPGKYTADGGKHVAYIIRSRVKDHYIFYSEGDCPGPVPGVWLVGRDPKNNLEALEDFEKAAGARGLSTESILIPRQSETSSPGSDSGGGGSLAEAKEAANAELDSYGVSDFYKRLIDKAKTVEGVEALKDAILAALPSAWSHPQFEK

SEQ ID NO: 9 - protein, 403 aa, artificial
  fusion protein
ASDEEIQDVSGTWYLKAMTVDFWCSGIHEESVTPMTLTTLEGGNLEAKVTMDIEGFLQEFKAVLEKTDEPGKYTADGGKHVAYIIRSRVKDHYIFYSEGDCPGPVPGVWLVGRDPKNNLEALEDFEKAAGARGLSTESILIPRQSETSSPGSDGGGGSGGGGSQDSTSDLIPAPPLSKVPLQQNFQDNQFHGKWYVVGEAGNLLLREDKDPRKMTATIYELKEDKSYDVTRVEFGAKTYKYQIGTFVPGSQPGEFTLGGIESMPGMTSFLVRVVSTNYNQHAIVFFKYVYQNREYFEITLYGRTKELTSELKENFIRFSKSLGLPENHIVFPVPIDQAIDGSGGGGSLAEAKEAANAELDSYGVSDFYKRLIDKAKTVEGVEALKDAILAALPSAWSHPQFEK

SEQ ID NO: 10 - protein, 378 aa, artificial
  fusion protein
ASDEEIQDVSGTWYLKAMTVDFWCSGIHEESVTPMTLTTLEGGNLEAKVTMDIEGFLQEFKAVLEKTDEPGKYTADGGKHVAYIIRSRVKDHYIFYSEGDCPGPVPGVWLVGRDPKNNLEALEDFEKAAGARGLSTESILIPRQSETSSPGSDGGGGSGGGGSASDEEIQDVSGTWYLKAMTVDFWCSGIHEESVTPMTLTTLEGGNLEAKVTMDIEGFLQEFKAVLEKTDEPGKYTADGGKHVAYIIRSRVKDHYIFYSEGDCPGPVPGVWLVGRDPKNNLEALEDFEKAAGARGLSTESILIPRQSETSSPGSDSGGGGSLAEAKEAANAELDSYGVSDFYKRLIDKAKTVEGVEALKDAILAALPSAWSHPQFEK

SEQ ID NO: 11 - protein, 390 aa, artificial
  fusion protein
DKTHTCPPCPAPELLGGPSVFLFPPKPKDTLMISRTPEVTCVVVDVSHEDPEVKFNWYVDGVEVHNAKTKPREEQYNSTYRVVSVLTVLHQDWLNGKEYKCKVSNKALPAPIEKTISKAKGQPREPQVYTLPPSREEMTKNQVSLTCLVKGFYPSDIAVEWESNGQPENNYKTTPPVLDSDGSFFLYSKLTVDKSRWQQGNVFSCSVMHEALHNHYTQKSLSLSPGKGGGGSGGGGSASDEEIQDVSGTWYLKAMTVDFWCSGIHEESVTPMTLTTLEGGNLEAKVTMDIEGFLQEFKAVLEKTDEPGKYTADGGKHVAYIIRSRVKDHYIFYSEGDCPGPVPGVWLVGRDPKNNLEALEDFEKAAGARGLSTESILIPRQSETSSPGSD

SEQ ID NO: 12 - protein, 553 aa, artificial
  fusion protein
ASDEEIQDVSGTWYLKAMTVDFWCSGIHEESVTPMTLTTLEGGNLEAKVTMDIEGFLQEFKAVLEKTDEPGKYTADGGKHVAYIIRSRVKDHYIFYSEGDCPGPVPGVWLVGRDPKNNLEALEDFEKAAGARGLSTESILIPRQSETSSPGSDGGGGSGGGGSDKTHTCPPCPAPELLGGPSVFLFPPKPKDTLMISRTPEVTCVVVDVSHEDPEVKFNWYVDGVEVHNAKTKPREEQYNSTYRVVSVLTVLHQDWLNGKEYKCKVSNKALPAPIEKTISKAKGQPREPQVYTLPPSREEMTKNQVSLTCLVKGFYPSDIAVEWESNGQPENNYKTTPPVLDSDGSFFLYSKLTVDKSRWQQGNVFSCSVMHEALHNHYTQKSLSLSPGKGGGGSGGGGSASDEEIQDVSGTWYLKAMTVDFWCSGIHEESVTPMTLTTLEGGNLEAKVTMDIEGFLQEFKAVLEKTDEPGKYTADGGKHVAYIIRSRVKDHYIFYSEGDCPGPVPGVWLVGRDPKNNLEALEDFEKAAGARGLSTESILIPRQSETSSPGSD

SEQ ID NO: 13 - protein, 553 aa, artificial
  fusion protein
DKTHTCPPCPAPELLGGPSVFLFPPKPKDTLMISRTPEVTCVVVDVSHEDPEVKFNWYVDGVEVHNAKTKPREEQYNSTYRVVSVLTVLHQDWLNGKEYKCKVSNKALPAPIEKTISKAKGQPREPQVYTLPPSREEMTKNQVSLTCLVKGFYPSDIAVEWESNGQPENNYKTTPPVLDSDGSFFLYSKLTVDKSRWQQGNVFSCSVMHEALHNHYTQKSLSLSPGKGGGGSGGGGSASDEEIQDVSGTWYLKAMTVDFWCSGIHEESVTPMTLTTLEGGNLEAKVTMDIEGFLQEFKAVLEKTDEPGKYTADGGKHVAYIIRSRVKDHYIFYSEGDCPGPVPGVWLVGRDPKNNLEALEDFEKAAGARGLSTESILIPRQSETSSPGSDGGGGSGGGGSASDEEIQDVSGTWYLKAMTVDFWCSGIHEESVTPMTLTTLEGGNLEAKVTMDIEGFLQEFKAVLEKTDEPGKYTADGGKHVAYIIRSRVKDHYIFYSEGDCPGPVPGVWLVGRDPKNNLEALEDFEKAAGARGLSTESILIPRQSETSSPGSD

SEQ ID NO: 14 - protein, 55 aa, artificial
  albumin binding domain
SAGAVDANSLAEAKVLANRELDKYGVSDYYKNLINNAKTVEGVKALIDEILAALP

SEQ ID NO: 15 - protein, 52 aa, artificial
  albumin binding domain
SGGGGSLAEAKEAANAELDSYGVSDFYKRLIDKAKTVEGVEALKDAILAALP

SEQ ID NO: 16 - protein, 227 aa, artificial
  Fc portion
DKTHTCPPCPAPELLGGPSVFLFPPKPKDTLMISRTPEVTCVVVDVSHEDPEVKFNWYVDGVEVHNAKTKPREEQYNSTYRVVSVLTVLHQDWLNGKEYKCKVSNKALPAPIEKTISKAKGQPREPQVYTLPPSREEMTKNQVSLTCLVKGFYPSDIAVEWESNGQPENNYKTTPPVLDSDGSFFLYSKLTVDKSRWQQGNVFSCSVMHEALHNHYTQKSLSLSPGK

SEQ ID NO: 17 - protein, 10 aa, artificial
  protein tag
SAWSHPQFEK

SEQ ID NO: 18 - protein, 12 aa, artificial
  synthetic linker
SDGGGGSGGGGS

SEQ ID NO: 19 - protein, 10 aa, artificial
  synthetic linker
GGGGSGGGGS

SEQ ID NO: 20 - protein, 2 aa, artificial
  synthetic linker
SD

SEQ ID NO: 21 - DNA, 453 bp, artificial
  lipocalin mutein
gcctcagacgaggagattcaggatgtgtcagggacgtggtatctgaaggccatgacggtggatttttggtgttctgggattcatgaggagtctgttacgccaatgactctgactacccttgaaggcggcaatctggaggctaaggtcaccatggatattgagggatttcttcaagagtttaaggcagtgttagagaagacagatgaaccgggtaaatatacggccgatggcggtaaacatgttgcctatatcattcgcagccgtgtgaaagatcattacatcttttatagcgagggagattgtcctggtccggttccaggggtgtggctcgtgggcagagaccccaagaacaacctggaagccttggaggactttgagaaagccgcaggagcccgcggactcagcacggagagcatcctcatccccaggcagagcgaaaccagctctccaggg

SEQ ID NO: 22 - DNA, 534 bp, artificial
  lipocalin mutein
caggactccacctcagacctgatcccagccccacctctgagcaaggtccctctgcagcagaacttccaggacaaccaattccatgggaaatggtatgtcgtgggcgaggccggaaatcttttgctgcgtgaggataaggatccgaggaaaatgacggcgaccatttacgagttgaaagaagataaatcatatgacgtcacccgggtggagtttggggctaagacatacaagtaccagattgggacctttgtgccggggagccagccgggcgagtttactttaggcggtattgaaagtatgccgggcatgacatcatttttggtccgtgtcgtgagcaccaactacaaccagcatgccatagtgttcttcaagtatgtgtatcagaaccgcgagtattttgagatcacactgtacgggcgcacgaaagaactgacaagcgagctgaaggaaaattttatccgcttttccaaatctctgggcctccctgaaaaccacatcgtcttccctgtcccaatcgaccaggctatcgacggc

SEQ ID NO: 23 - DNA, 1053 bp, artificial
  fusion protein
gcctcagacgaggagattcaggatgtgtcagggacgtggtatctgaaggccatgacggtggatttttggtgttctgggattcatgaggagtctgttacgccaatgactctgactacccttgaaggcggcaatctggaggctaaggtcaccatggatattgagggatttcttcaagagtttaaggcagtgttagagaagacagatgaaccgggtaaatatacggccgatggcggtaaacatgttgcctatatcattcgcagccgtgtgaaagatcattacatcttttatagcgagggagattgtcctggtccggttccaggggtgtggctcgtgggcagagaccccaagaacaacctggaagccttggaggactttgagaaagccgcaggagcccgcggactcagcacggagagcatcctcatccccaggcagagcgaaaccagctctccagggagcgacggtggtggtggttctggtggtggtggatcgcaggactccacctcagacctgatcccagccccacctctgagcaaggtccctctgcagcagaacttccaggacaaccaattccatgggaaatggtatgtcgtgggcgaggccggaaatcttttgctgcgtgaggataaggatccgaggaaaatgacggcgaccatttacgagttgaaagaagataaatcatatgacgtcacccgggtggagtttggggctaagacatacaagtaccagattgggacctttgtgccggggagccagccgggcgagtttactttaggcggtattgaaagtatgccgggcatgacatcatttttggtccgtgtcgtgagcaccaactacaaccagcatgccatagtgttcttcaagtatgtgtatcagaaccgcgagtattttgagatcacactgtacgggcgcacgaaagaactgacaagcgagctgaaggaaaattttatccgcttttccaaatctctgggcctccctgaaaaccacatcgtcttccctgtcccaatcgaccaggctatcgacggcagcgcttggtctcacccgcagttcgaaaaa

SEQ ID NO: 24 - DNA, 1047 bp, artificial
  fusion protein
caggactccacctcagacctgatcccagccccacctctgagcaaggtccctctgcagcagaacttccaggacaaccaattccatgggaaatggtatgtcgtgggcgaggccggaaatcttttgctgcgtgaggataaggatccgaggaaaatgacggcgaccatttacgagttgaaagaagataaatcatatgacgtcacccgggtggagtttggggctaagacatacaagtaccagattgggacctttgtgccggggagccagccgggcgagtttactttaggcggtattgaaagtatgccgggcatgacatcatttttggtccgtgtcgtgagcaccaactacaaccagcatgccatagtgttcttcaagtatgtgtatcagaaccgcgagtattttgagatcacactgtacgggcgcacgaaagaactgacaagcgagctgaaggaaaattttatccgcttttccaaatctctgggcctccctgaaaaccacatcgtcttccctgtcccaatcgaccaggctatcgacggcggcggtggtggttctggtggtggtggatcggcctcagacgaggagattcaggatgtgtcagggacgtggtatctgaaggccatgacggtggatttttggtgttctgggattcatgaggagtctgttacgccaatgactctgactacccttgaaggcggcaatctggaggctaaggtcaccatggatattgagggatttcttcaagagtttaaggcagtgttagagaagacagatgaaccgggtaaatatacggccgatggcggtaaacatgttgcctatatcattcgcagccgtgtgaaagatcattacatcttttatagcgagggagattgtcctggtccggttccaggggtgtggctcgtgggcagagaccccaagaacaacctggaagccttggaggactttgagaaagccgcaggagcccgcggactcagcacggagagcatcctcatccccaggcagagcgaaaccagctctccagggagcgcttggtctcacccgcagttcgaaaaa

SEQ ID NO: 25 - DNA, 1218 bp, artificial
  fusion protein
gcctcagacgaggagattcaggatgtgtcagggacgtggtatctgaaggccatgacggtggatttttggtgttctgggattcatgaggagtctgttacgccaatgactctgactacccttgaaggcggcaatctggaggctaaggtcaccatggatattgagggatttcttcaagagtttaaggcagtgttagagaagacagatgaaccgggtaaatatacggccgatggcggtaaacatgttgcctatatcattcgcagccgtgtgaaagatcattacatcttttatagcgagggagattgtcctggtccggttccaggggtgtggctcgtgggcagagaccccaagaacaacctggaagccttggaggactttgagaaagccgcaggagcccgcggactcagcacggagagcatcctcatccccaggcagagcgaaaccagctctccagggagcgacggtggtggtggttctggtggtggtggatcgcaggactccacctcagacctgatcccagccccacctctgagcaaggtccctctgcagcagaacttccaggacaaccaattccatgggaaatggtatgtcgtgggcgaggccggaaatcttttgctgcgtgaggataaggatccgaggaaaatgacggcgaccatttacgagttgaaagaagataaatcatatgacgtcacccgggtggagtttggggctaagacatacaagtaccagattgggacctttgtgccggggagccagccgggcgagtttactttaggcggtattgaaagtatgccgggcatgacatcatttttggtccgtgtcgtgagcaccaactacaaccagcatgccatagtgttcttcaagtatgtgtatcagaaccgcgagtattttgagatcacactgtacgggcgcacgaaagaactgacaagcgagctgaaggaaaattttatccgcttttccaaatctctgggcctccctgaaaaccacatcgtcttccctgtcccaatcgaccaggctatcgacggcagcgctggtgccgtcgacgctaactctctggctgaagctaaagttctggctaaccgtgaactggacaaatacggtgtttccgactactacaaaaacctcatcaacaacgctaaaaccgttgaaggtgttaaagctctgatcgacgaaattctcgcagcactgccgagcgcttggtctcacccgcagttcgaaaaa

SEQ ID NO: 26 - DNA, 1671 bp, artificial
  fusion protein
gcaagtgatgaagaaattcaggatgttagcggcacctggtatctgaaagcaatgaccgttgatttttggtgcagcggtattcatgaagaaagcgttaccccgatgaccctgaccaccctggaaggtggtaatctggaagcaaaagttaccatggatattgagggttttctgcaagaatttaaagccgtgctggaaaaaaccgatgaaccgggtaaatataccgcagatggtggtaaacatgtggcctatattatccgtagccgtgtgaaagatcactatatcttttatagcgaaggtgattgtccgggtccggttccgggtgtttggctggttggtcgtgatccgaaaaataacctggaagcactggaagattttgaaaaagcagccggtgcacgtggtctgagcaccgaaagcattctgattccgcgtcagagcgaaaccagcagtcctggatccgacggtggtggtggttctggtggtggtggatcggcctcagacgaggagattcaggatgtgtcagggacgtggtatctgaaggccatgacggtggatttttggtgttctgggattcatgaggagtctgttacgccaatgactctgactacccttgaaggcggcaatctggaggctaaggtcaccatggatattgagggatttcttcaagagtttaaggcagtgttagagaagacagatgaaccgggtaaatatacggccgatggcggtaaacatgttgcctatatcattcgcagccgtgtgaaagatcattacatcttttatagcgagggagattgtcctggtccggttccaggggtgtggctcgtgggcagagaccccaagaacaacctggaagccttggaggactttgagaaagccgcaggagcccgcggactcagcacggagagcatcctcatccccaggcagagcgaaaccagctctccagggagcgacggcggaggtggctcaggaggtggcggatcccaggactccacctcagacctgatcccagccccacctctgagcaaggtccctctgcagcagaacttccaggacaaccaattccatgggaaatggtatgtcgtgggcgaggccggaaatcttttgctgcgtgaggataaggatccgaggaaaatgacggcgaccatttacgagttgaaagaagataaatcatatgacgtcacccgggtggagtttggggctaagacatacaagtaccagattgggacctttgtgccggggagccagccgggcgagtttactttaggcggtattgaaagtatgccgggcatgacatcatttttggtccgtgtcgtgagcaccaactacaaccagcatgccatagtgttcttcaagtatgtgtatcagaaccgcgagtattttgagatcacactgtacgggcgcacgaaagaactgacaagcgagctgaaggaaaattttatccgcttttccaaatctctgggcctccctgaaaaccacatcgtcttccctgtcccaatcgaccaggctatcgacggcagcggcggcggcggctctctggctgaagctaaagaagcggctaacgcggaactggactcttacggtgtttccgacttttacaaacgtctcatcgataaagctaaaaccgttgaaggtgttgaagctctgaaagacgcgattctcgcagcactgccgaaa

SEQ ID NO: 27 - DNA, 720 bp, artificial
  fusion protein
caggactccacctcagacctgatcccagccccacctctgagcaaggtccctctgcagcagaacttccaggacaaccaattccatgggaaatggtatgtcgtgggcgaggccggaaatcttttgctgcgtgaggataaggatccgaggaaaatgacggcgaccatttacgagttgaaagaagataaatcatatgacgtcacccgggtggagtttggggctaagacatacaagtaccagattgggacctttgtgccggggagccagccgggcgagtttactttaggcggtattgaaagtatgccgggcatgacatcatttttggtccgtgtcgtgagcaccaactacaaccagcatgccatagtgttcttcaagtatgtgtatcagaaccgcgagtattttgagatcacactgtacgggcgcacgaaagaactgacaagcgagctgaaggaaaattttatccgcttttccaaatctctgggcctccctgaaaaccacatcgtcttccctgtcccaatcgaccaggctatcgacggcagcggcggcggcggctctctggctgaagctaaagaagcggctaacgcggaactggactcttacggtgtttccgacttttacaaacgtctcatcgataaagctaaaaccgttgaaggtgttgaagctctgaaagacgcgattctcgcagcactgccgagcgcttggtctcacccgcagttcgaaaaa

SEQ ID NO: 28 - DNA, 645 bp, artificial
  fusion protein
gcctcagacgaggagattcaggatgtgtcagggacgtggtatctgaaggccatgacggtggatttttggtgttctgggattcatgaggagtctgttacgccaatgactctgactacccttgaaggcggcaatctggaggctaaggtcaccatggatattgagggatttcttcaagagtttaaggcagtgttagagaagacagatgaaccgggtaaatatacggccgatggcggtaaacatgttgcctatatcattcgcagccgtgtgaaagatcattacatcttttatagcgagggagattgtcctggtccggttccaggggtgtggctcgtgggcagagaccccaagaacaacctggaagccttggaggactttgagaaagccgcaggagcccgcggactcagcacggagagcatcctcatccccaggcagagcgaaaccagctctccagggagcgatagcggcggcggcggctctctggctgaagctaaagaagcggctaacgcggaactggactcttacggtgtttccgacttttacaaacgtctcatcgataaagctaaaaccgttgaaggtgttgaagctctgaaagacgcgattctcgcagcactgccgagcgcttggtctcacccgcagttcgaaaaa

SEQ ID NO: 29 - DNA, 1209 bp, artificial
  fusion protein
gcctcagacgaggagattcaggatgtgtcagggacgtggtatctgaaggccatgacggtggatttttggtgttctgggattcatgaggagtctgttacgccaatgactctgactacccttgaaggcggcaatctggaggctaaggtcaccatggatattgagggatttcttcaagagtttaaggcagtgttagagaagacagatgaaccgggtaaatatacggccgatggcggtaaacatgttgcctatatcattcgcagccgtgtgaaagatcattacatcttttatagcgagggagattgtcctggtccggttccaggggtgtggctcgtgggcagagaccccaagaacaacctggaagccttggaggactttgagaaagccgcaggagcccgcggactcagcacggagagcatcctcatccccaggcagagcgaaaccagctctccagggagcgacggcggaggtggctcaggaggtggcggatcccaggactccacctcagacctgatcccagccccacctctgagcaaggtccctctgcagcagaacttccaggacaaccaattccatgggaaatggtatgtcgtgggcgaggccggaaatcttttgctgcgtgaggataaggatccgaggaaaatgacggcgaccatttacgagttgaaagaagataaatcatatgacgtcacccgggtggagtttggggctaagacatacaagtaccagattgggacctttgtgccggggagccagccgggcgagtttactttaggcggtattgaaagtatgccgggcatgacatcatttttggtccgtgtcgtgagcaccaactacaaccagcatgccatagtgttcttcaagtatgtgtatcagaaccgcgagtattttgagatcacactgtacgggcgcacgaaagaactgacaagcgagctgaaggaaaattttatccgcttttccaaatctctgggcctccctgaaaaccacatcgtcttccctgtcccaatcgaccaggctatcgacggcagcggcggcggcggctctctggctgaagctaaagaagcggctaacgcggaactggactcttacggtgtttccgacttttacaaacgtctcatcgataaagctaaaaccgttgaaggtgttgaagctctgaaagacgcgattctcgcagcactgccgagcgcttggtctcacccgcagttcgaaaaa

SEQ ID NO: 30 - DNA, 1134 bp, artificial
  fusion protein
gcaagtgatgaagaaattcaggatgttagcggcacctggtatctgaaagcaatgaccgttgatttttggtgcagcggtattcatgaagaaagcgttaccccgatgaccctgaccaccctggaaggtggtaatctggaagcaaaagttaccatggatattgagggttttctgcaagaatttaaagccgtgctggaaaaaaccgatgaaccgggtaaatataccgcagatggtggtaaacatgtggcctatattatccgtagccgtgtgaaagatcactatatcttttatagcgaaggtgattgtccgggtccggttccgggtgtttggctggttggtcgtgatccgaaaaataacctggaagcactggaagattttgaaaaagcagccggtgcacgtggtctgagcaccgaaagcattctgattccgcgtcagagcgaaaccagcagtcctggatccgacggtggtggtggttctggtggtggtggatcggcctcagacgaggagattcaggatgtgtcagggacgtggtatctgaaggccatgacggtggatttttggtgttctgggattcatgaggagtctgttacgccaatgactctgactacccttgaaggcggcaatctggaggctaaggtcaccatggatattgagggatttcttcaagagtttaaggcagtgttagagaagacagatgaaccgggtaaatatacggccgatggcggtaaacatgttgcctatatcattcgcagccgtgtgaaagatcattacatcttttatagcgagggagattgtcctggtccggttccaggggtgtggctcgtgggcagagaccccaagaacaacctggaagccttggaggactttgagaaagccgcaggagcccgcggactcagcacggagagcatcctcatccccaggcagagcgaaaccagctctccagggagcgatagcggcggcggcggctctctggctgaagctaaagaagcggctaacgcggaactggactcttacggtgtttccgacttttacaaacgtctcatcgataaagctaaaaccgttgaaggtgttgaagctctgaaagacgcgattctcgcagcactgccgagcgcttggtctcacccgcagttcgaaaaa

SEQ ID NO: 31 - DNA, 1173 bp, artificial
  fusion protein
gacaaaacccacacctgcccaccttgtcctgcccctgaactgctgggaggaccttctgtgtttctgttcccaccaaaaccaaaagataccctgatgatctctagaacccctgaggtgacatgtgtggtggtggatgtgtctcatgaggaccctgaggtcaaattcaactggtacgtggatggagtggaagtccacaatgccaaaaccaagcctagagaggaacagtacaattcaacctacagagtggtcagtgtgctgactgtgctgcatcaggattggctgaatggcaaggaatacaagtgtaaagtctcaaacaaggccctgcctgctccaattgagaaaacaatctcaaaggccaagggacagcctagggaaccccaggtctacaccctgccaccttcaagagaggaaatgaccaaaaaccaggtgtccctgacatgcctggtcaaaggcttctacccttctgacattgctgtggagtgggagtcaaatggacagcctgagaacaactacaaaacaaccccccctgtgctggattctgatggctctttctttctgtactccaaactgactgtggacaagtctagatggcagcaggggaatgtcttttcttgctctgtcatgcatgaggctctgcataaccactacactcagaaatccctgtctctgtctcctggcaaaggcggcggaggatccggcggaggaggtagcgcatcagacgaggaaatccaggacgtgtcagggacctggtacctgaaagccatgaccgtggatttttggtgctccggcatccatgaggagtcagtcactcccatgaccctgacaaccctagaaggtgggaatctggaggccaaagtgacaatggatattgagggctttctccaggagttcaaagccgtcctcgagaagacagacgagcctggaaagtatactgctgatgggggaaaacacgtagcctatatcattcgatctcgggtgaaggatcattatatcttctattccgagggcgactgccccggccctgtgccaggtgtctggctagttgggagggaccccaagaacaatctcgaggctctggaggacttcgagaaggcagctggtgccaggggattgagcactgagtctatccttatcccacgccagagcgagacctcaagcccagggtccgactga

SEQ ID NO: 32 - DNA, 1659 bp, artificial
  fusion protein
gcatcagacgaggaaatccaggacgtgtcagggacctggtacctgaaagccatgaccgtggatttttggtgctccggcatccatgaggagtcagtcactcccatgaccctgacaaccctagaaggtgggaatctggaggccaaagtgacaatggatattgagggctttctccaggagttcaaagccgtcctcgagaagacagacgagcctggaaagtatactgctgatgggggaaaacacgtagcctatatcattcgatctcgggtgaaggatcattatatcttctattccgagggcgactgccccggccctgtgccaggtgtctggctagttgggagggaccccaagaacaatctcgaggctctggaggacttcgagaaggcagctggtgccaggggattgagcactgagtctatccttatcccacgccagagcgagacctcaagcccagggtccgacggcggtggaggatccggtggaggcggttctgacaaaacccacacctgcccaccttgtcctgcccctgaactgctgggaggaccttctgtgtttctgttcccaccaaaaccaaaagataccctgatgatctctagaacccctgaggtgacatgtgtggtggtggatgtgtctcatgaggaccctgaggtcaaattcaactggtacgtggatggagtggaagtccacaatgccaaaaccaagcctagagaggaacagtacaattcaacctacagagtggtcagtgtgctgactgtgctgcatcaggattggctgaatggcaaggaatacaagtgtaaagtctcaaacaaggccctgcctgctccaattgagaaaacaatctcaaaggccaagggacagcctagggaaccccaggtctacaccctgccaccttcaagagaggaaatgaccaaaaaccaggtgtccctgacatgcctggtcaaaggcttctacccttctgacattgctgtggagtgggagtcaaatggacagcctgagaacaactacaaaacaaccccccctgtgctggattctgatggctctttctttctgtactccaaactgactgtggacaagtctagatggcagcaggggaatgtcttttcttgctctgtcatgcatgaggctctgcataaccactacactcagaaatccctgtctctgtctcccgggaaagggggtgggggatccggcggaggaggtagcgcatcagacgaggaaatccaggacgtgtcagggacctggtacctgaaagccatgaccgtggatttttggtgctccggcatccatgaggagtcagtcactcccatgaccctgacaaccctagaaggtgggaatctggaggccaaagtgacaatggatattgagggctttctccaggagttcaaagccgtcctcgagaagacagacgagcctggaaagtatactgctgatgggggaaaacacgtagcctatatcattcgatctcgggtgaaggatcattatatcttctattccgagggcgactgccccggccctgtgccaggtgtctggctagttgggagggaccccaagaacaatctcgaggctctggaggacttcgagaaggcagctggtgccaggggattgagcactgagtctatccttatcccacgccagagcgagacctcaagcccagggtccgac

SEQ ID NO: 33 - DNA, 1659 bp, artificial
  fusion protein
gacaaaacccacacctgcccaccttgtcctgcccctgaactgctgggaggaccttctgtgtttctgttcccaccaaaaccaaaagataccctgatgatctctagaacccctgaggtgacatgtgtggtggtggatgtgtctcatgaggaccctgaggtcaaattcaactggtacgtggatggagtggaagtccacaatgccaaaaccaagcctagagaggaacagtacaattcaacctacagagtggtcagtgtgctgactgtgctgcatcaggattggctgaatggcaaggaatacaagtgtaaagtctcaaacaaggccctgcctgctccaattgagaaaacaatctcaaaggccaagggacagcctagggaaccccaggtctacaccctgccaccttcaagagaggaaatgaccaaaaaccaggtgtccctgacatgcctggtcaaaggcttctacccttctgacattgctgtggagtgggagtcaaatggacagcctgagaacaactacaaaacaaccccccctgtgctggattctgatggctctttctttctgtactccaaactgactgtggacaagtctagatggcagcaggggaatgtcttttcttgctctgtcatgcatgaggctctgcataaccactacactcagaaatccctgtctctgtctcctggcaaaggcggcggaggatccggcggaggaggtagcgcatcagacgaggaaatccaggacgtgtcagggacctggtacctgaaagccatgaccgtggatttttggtgctccggcatccatgaggagtcagtcactcccatgaccctgacaaccctagaaggtgggaatctggaggccaaagtgacaatggatattgagggctttctccaggagttcaaagccgtcctcgagaagacagacgagcctggaaagtatactgctgatgggggaaaacacgtagcctatatcattcgatctcgggtgaaggatcattatatcttctattccgagggcgactgccccggccctgtgccaggtgtctggctagttgggagggaccccaagaacaatctcgaggctctggaggacttcgagaaggcagctggtgccaggggattgagcactgagtctatccttatcccacgccagagcgagacctcaagcccagggtccgacggcggcggtgggtccggcggcggtggctccgcgtccgatgaagaaatccaggatgtgagcggcacctggtatctgaaagcaatgaccgttgacttctggtgctccggcatccatgaagaaagcgtgaccccaatgaccttgaccacgctggaaggcggtaatttagaagccaaagtaactatggatatcgaaggcttcctgcaggaatttaaagcggtgctggaaaaaactgatgagccaggtaaatacaccgccgacggtggcaaacacgtggcctatattatccgttctcgtgtcaaagaccattatatcttctactctgaaggcgattgccccggtccggttccgggcgtctggcttgtcggtcgtgacccgaaaaacaacctggaagcactcgaagacttcgaaaaagcggcaggcgcgcgtggtctgtctaccgagagcatccttatcccacgtcagagcgaaacctccagccctggttccgat

SEQ ID NO: 34 - DNA, 165 bp, artificial
  albumin binding domain
agcgctggtgccgtcgacgctaactctctggctgaagctaaagttctggctaaccgtgaactggacaaatacggtgtttccgactactacaaaaacctcatcaacaacgctaaaaccgttgaaggtgttaaagctctgatcgacgaaattctcgcagcactgccg

SEQ ID NO: 35 - DNA, 156 bp, artificial
  albumin binding domain
agcggcggcggcggctctctggctgaagctaaagaagcggctaacgcggaactggactcttacggtgtttccgacttttacaaacgtctcatcgataaagctaaaaccgttgaaggtgttgaagctctgaaagacgcgattctcgcagcactgccg

SEQ ID NO: 36 - DNA, 681 bp, artificial
  Fc portion
gacaaaacccacacctgcccaccttgtcctgcccctgaactgctgggaggaccttctgtgtttctgttcccaccaaaaccaaaagataccctgatgatctctagaacccctgaggtgacatgtgtggtggtggatgtgtctcatgaggaccctgaggtcaaattcaactggtacgtggatggagtggaagtccacaatgccaaaaccaagcctagagaggaacagtacaattcaacctacagagtggtcagtgtgctgactgtgctgcatcaggattggctgaatggcaaggaatacaagtgtaaagtctcaaacaaggccctgcctgctccaattgagaaaacaatctcaaaggccaagggacagcctagggaaccccaggtctacaccctgccaccttcaagagaggaaatgaccaaaaaccaggtgtccctgacatgcctggtcaaaggcttctacccttctgacattgctgtggagtgggagtcaaatggacagcctgagaacaactacaaaacaaccccccctgtgctggattctgatggctctttctttctgtactccaaactgactgtggacaagtctagatggcagcaggggaatgtcttttcttgctctgtcatgcatgaggctctgcataaccactacactcagaaatccctgtctctgtctcctggcaag

SEQ ID NO: 37 - DNA, 30 bp, artificial
  protein tag
agcgcttggtctcacccgcagttcgaaaaa

SEQ ID NO: 38 - DNA, 36 bp, artificial
  synthetic linker
agcgacggtggtggtggttctggtggtggtggatcg

SEQ ID NO: 39 - DNA, 30 bp, artificial
  synthetic linker
ggtggtggtggttctggtggtggtggatcg

SEQ ID NO: 40 - DNA, 6 bp, artificial
  synthetic linker
agcgac

SEQ ID NO: 41 - protein, 152 aa, human
ASDEEIQDVSGTWYLKAMTVDREFPEMNLESVTPMTLTTLEGGNLEAKVTMLISGRCQEVKAVLEKTDEPGKYTADGGKHVAYIIRSHVKDHYIFYCEGELHGKPVRGVKLVGRDPKNNLEALEDFEKAAGARGLSTESILIPRQSETCSPG

SEQ ID NO: 42 - protein, 151 aa, artificial
  lipocalin mutein
ASDEEIQDVSGTWYLKAMTVDFWCSGIHEESVTPMTLTTLEGGNLEAKVTMDIEGFLQEFKAVLEKTDEPGKYTADGGKHVAYIIRSHVKDHYIFYSEGDCPGPVPGVWLVGRDPKNNLEALEDFEKAAGARGLSTESILIPRQSETSSPG

SEQ ID NO: 43 - protein, 178 aa, human
QDSTSDLIPAPPLSKVPLQQNFQDNQFQGKWYVVGLAGNAILREDKDPQKMYATIYELKEDKSYNVTSVLFRKKKCDYWIRTFVPGCQPGEFTLGNIKSYPGLTSYLVRVVSTNYNQHAMVFFKKVSQNREYFKITLYGRTKELTSELKENFIRFSKSLGLPENHIVFPVPIDQCIDG

SEQ ID NO: 44 - protein, 178 aa, artificial
  lipocalin mutein
QDSTSDLIPAPPLSKVPLQQNFQDNQFHGKWYVVGEAGNLLLREDKDPRKMTATIYELKEDKSYNVTRVEFGVKTYKYQIGTFVPGSQPGEFTLGGIKSMPGMTSFLVRVVSTNYNQHAMVFFKYVYQNREYFEITLYGRTKELTSELKENFIRFSKSLGLPENHIVFPVPIDQAIDG

SEQ ID NO: 45 - protein, 178 aa, artificial
  lipocalin mutein
QDSTSDLIPAPPLSKVPLQQNFQDNQFHGKWYVVGEAGNLILREDKDPRKMTATIYELKEDKSYDVTRVEFGVKTRKYRIGTFVPGSQPGEFTLGGIKSMPGMTSFLVRVVSTNYNQHAMVFFKYVYQNREYFEITLYGRTKELTSELKENFIRFSKSLGLPENHIVFPVPIDQAIDG

SEQ ID NO: 46 - protein, 178 aa, artificial
  lipocalin mutein
QDSTSDLIPAPPLSKVPLQQNFQDNQFHGKWYVVGEAGNLLLREDKDPRKMTATIYELREDKSYDVTRVEFGVKTYKYQIGTFVPGSQPGEFTLGGIKSMPGMTSFLVRVVSTDYNQHAMVFFKYVYQNREYFEITLYGRTKELTSELKENFIRFSKSLGLPENHIVFPVPIDQAIDG

SEQ ID NO: 47 - DNA, 456 bp, human
gcctcagacgaggagattcaggatgtgtcagggacgtggtatctgaaggccatgacggtggacagggagttccctgagatgaatctggaatcggtgacacccatgaccctcacgaccctggaagggggcaacctggaagccaaggtcaccatgctgataagtggccggtgccaggaggtgaaggccgtcctggagaaaactgacgagccgggaaaatacacggccgacgggggcaagcacgtggcatacatcatcaggtcgcacgtgaaggaccactacatcttttactgtgagggcgagctgcacgggaagccggtccgaggggtgaagctcgtgggcagagaccccaagaacaacctggaagccttggaggactttgagaaagccgcaggagcccgcggactcagcacggagagcatcctcatccccaggcagagcgaaacctgctctccaggg

SEQ ID NO: 48 - DNA, 453 bp, artificial
  lipocalin mutein
gcctcagacgaggagattcaggatgtgtcagggacgtggtatctgaaggccatgacggtggatttttggtgttctgggattcatgaggagtctgttacgccaatgactctgactacccttgaaggcggcaatctggaggctaaggtcaccatggatattgagggatttcttcaagagtttaaggcagtgttagagaagacagatgaaccgggtaaatatacggccgatggcggtaaacatgttgcctatatcattcgcagccatgtgaaagatcattacatcttttatagcgagggagattgtcctggtccggttccaggggtgtggctcgtgggcagagaccccaagaacaacctggaagccttggaggactttgagaaagccgcaggagcccgcggactcagcacggagagcatcctcatccccaggcagagcgaaaccagctctccaggg

SEQ ID NO: 49 - DNA, 534 bp, human
caggactccacctcagacctgatcccagccccacctctgagcaaggtccctctgcagcagaacttccaggacaaccaattccaggggaagtggtatgtggtaggcctggcagggaatgcaattctcagagaagacaaagacccgcaaaagatgtatgccaccatctatgagctgaaagaagacaagagctacaatgtcacctccgtcctgtttaggaaaaagaagtgtgactactggatcaggacttttgttccaggttgccagcccggcgagttcacgctgggcaacattaagagttaccctggattaacgagttacctcgtccgagtggtgagcaccaactacaaccagcatgctatggtgttctttaagaaagtttctcaaaacagggagtacttcaagatcaccctctacgggagaaccaaggagctgacttcggaactaaaggagaacttcatccgcttctccaaatctctgggcctccctgaaaaccacatcgtcttccctgtcccaatcgaccagtgtatcgacggc

SEQ ID NO: 50 - DNA, 534 bp, artificial
  lipocalin mutein
caggactccacctcagacctgatcccagccccacctctgagcaaggtccctctgcagcagaacttccaggacaaccaattccatgggaaatggtatgtcgtgggcgaggccggaaatcttttgctgcgtgaggataaggatccgaggaaaatgacggcgaccatttacgagttgaaagaagataaatcatataacgtcacccgggtggagtttggggttaagacatacaagtaccagattgggacctttgtgccggggagccagccgggcgagtttactttaggcggtattaaaagtatgccgggcatgacatcatttttggtccgcgtcgtgagcaccaactacaaccagcatgccatggtgttcttcaagtatgtgtatcagaaccgcgagtattttgagatcacactgtacgggcgcacgaaagaactgacaagcgagctgaaggaaaattttatccgcttttccaaatctctgggcctccctgaaaaccacatcgtcttccctgtcccaatcgaccaggctatcgacggc

SEQ ID NO: 51 - DNA, 534 bp, artificial
  lipocalin mutein
caggactccacctcagacctgatcccagccccacctctgagcaaggtccctctgcagcagaacttccaggacaaccaattccatgggaaatggtacgtagtaggtgaggccggaaatctgattctgcgtgaggataaggatccgagaaaaatgactgcgaccatttacgagttgaaagaagataaatcatatgacgtcaccagggtggagtttggggtgaagacgcgtaagtaccggattgggacctttgtgccggggagccagccgggcgagtttactttaggcggtattaaaagtatgccgggcatgacatcatttttggtccgcgtcgtgagcaccaactacaaccagcatgccatggtgttcttcaagtacgtgtatcagaaccgcgagtattttgagatcacactgtacgggcgcacgaaagaactgacaagcgagctgaaggaaaattttatccgcttttccaaatctctgggcctccctgaaaaccacatcgtcttccctgtcccaatcgaccaggctatcgacggc

SEQ ID NO: 52 - DNA, 534 bp, artificial
  lipocalin mutein
caggactccacctcagacctgatcccagccccacctctgagcaaggtccctctgcagcagaacttccaggacaaccaattccatgggaaatggtatgtcgtgggcgaggccggaaatcttttgctgcgtgaggataaggatccgaggaaaatgacggcgaccatttacgagttgagagaagataaatcatatgacgtcacccgggtggagtttggggttaagacatacaagtaccagattgggacctttgtgccggggagccagccgggcgagtttactttaggcggtattaaaagtatgccgggcatgacatcatttttggtccgcgtcgtgagcaccgactacaaccagcatgccatggtgttcttcaagtatgtgtatcagaaccgcgagtattttgagatcacactgtacgggcgcacgaaagaactgacaagcgagttgaaggaaaattttatccgcttttccaaatctctgggcctccctgaaaaccacatcgtcttccctgtcccaatcgaccaggctatcgacggc

SEQ ID NO: 53 - protein, 457 aa, artificial
  reference antibody heavy chain
EVQLVESGGGLVQPGGSLRLSCAASGFTFSNYWMNWVRQAPGKGLEWVAAINQDGSEKYYVGSVKGRFTISRDNAKNSLYLQMNSLRVEDTAVYYCVRDYYDILTDYYIHYWYFDLWGRGTLVTVSSASTKGPSVFPLAPSSKSTSGGTAALGCLVKDYFPEPVTVSWNSGALTSGVHTFPAVLQSSGLYSLSSVVTVPSSSLGTQTYICNVNHKPSNTKVDKKVEPKSCDKTHTCPPCPAPELLGGPSVFLFPPKPKDTLMISRTPEVTCVVVDVSHEDPEVKFNWYVDGVEVHNAKTKPREEQYNSTYRVVSVLTVLHQDWLNGKEYKCKVSNKALPAPIEKTISKAKGQPREPQVYTLPPSREEMTKNQVSLTCLVKGFYPSDIAVEWESNGQPENNYKTTPPVLDSDGSFFLYSKLTVDKSRWQQGNVFSCSVMHEALHNHYTQKSLSLSPGK

SEQ ID NO: 54 - protein, 215 aa, artificial
  reference antibody light chain
EIVLTQSPGTLSLSPGERATLSCRASQSVSSSYLAWYQQKPGQAPRLLIYGASSRATGIPDRFSGSGSGTDFTLTISRLEPEDFAVYYCQQYGSSPCTFGQGTRLEIKRTVAAPSVFIFPPSDEQLKSGTASVVCLLNNFYPREAKVQWKVDNALQSGNSQESVTEQDSKDSTYSLSSTLTLSKADYEKHKVYACEVTHQGLSSPVTKSFNRGEC

SEQ ID NO: 55 - protein, 446 aa, artificial
  reference antibody heavy chain
QVQLVQSGAEVKKPGSSVKVSCKASGYSFTDYHISWVRQAPGQGLEWMGVINPEYGTTDYNQRFKGRVTITADESTSTAYMELSSLRSEDTAVYYCARYDYFTGTGAYWGQGTLVTVSSASTKGPSVFPLAPCSRSTSESTAALGCLVKDYFPEPVTVSWNSGALTSGVHTFPAVLQSSGLYSLSSVVTVPSSSLGTKTYTCNVDHKPSNTKVDKRVESKYGPPCPSCPAPEFLGGPSVFLFPPKPKDTLMISRTPEVTCVVVDVSQEDPEVQFNWYVDGVEVHNAKTKPREEQFNSTYRVVSVLTVLHQDWLNGKEYKCKVSNKGLPSSIEKTISKAKGQPREPQVYTLPPSQEEMTKNQVSLTCLVKGFYPSDIAVEWESNGQPENNYKTTPPVLDSDGSFFLYSRLTVDKSRWQEGNVFSCSVMHEALHNHYTQKSLSLSLGK

SEQ ID NO: 56 - protein, 219 aa, artificial
  reference antibody light chain
DIVMTQTPLSLSVTPGQPASISCRSSQSLKHSRGNTFLHWYLQKPGQSPQLLIYKVSNRFIGVPDRFSGSGSGTDFTLKISRVEAEDVGVYYCSQSTHYPFTFGQGTKLEIKRTVAAPSVFIFPPSDEQLKSGTASVVCLLNNFYPREAKVQWKVDNALQSGNSQESVTEQDSKDSTYSLSSTLTLSKADYEKHKVYACEVTHQGLSSPVTKSFNRGEC

SEQ ID NO: 57 - protein, 449 aa, artificial
  reference antibody heavy chain
QVQLVQSGAEVKKPGASVKVSCKVSGKTFWSYGINWVRQAPGKGLEWMGYIYIGTGYTEPNPKYKGRVTMTEDTSTDTAYMELSSLRSEDTAVYYCATIGGYYGNFDQWGQGTTVTVSSASTKGPSVFPLAPSSKSTSGGTAALGCLVKDYFPEPVTVSWNSGALTSGVHTFPAVLQSSGLYSLSSVVTVPSSSLGTQTYICNVNHKPSNTKVDKKVEPKSCDKTHTCPPCPAPELLGGPSVFLFPPKPKDTLMISRTPEVTCVVVDVSHEDPEVKFNWYVDGVEVHNAKTKPREEQYNSTYRVVSVLTVLHQDWLNGKEYKCKVSNKALPAPIEKTISKAKGQPREPQVYTLPPSRDELTKNQVSLTCLVKGFYPSDIAVEWESNGQPENNYKTTPPVLDSDGSFFLYSKLTVDKSRWQQGNVFSCSVMHEALHNHYTQKSLSLSPGK

SEQ ID NO: 58 - protein, 219 aa, artificial
  reference antibody light chain
DVVMTQSPLSLPVTLGQPASISCRSSQSLLISGGKTYLNWFQQRPGQSPRRLIYLVSKLDQGVPDRFSGSGSGTDFTLKISRVEAEDVGVYYCWQGTYFPLTFGQGTKLEIKRTVAAPSVFIFPPSDEQLKSGTASVVCLLNNFYPREAKVQWKVDNALQSGNSQESVTEQDSKDSTYSLSSTLTLSKADYEKHKVYACEVTHQGLSSPVTKSFNRGEC

SEQ ID NO: 59 - protein, 447 aa, artificial
  reference antibody heavy chain
EVQLVQSGAEVKKPGESLKISCKGSGYSFSNYWIGWVRQMPGKGLEWMGIIDPSNSYTRYSPSFQGQVTISADKSISTAYLQWSSLKASDTAMYYCARWYYKPFDVWGQGTLVTVSSASTKGPSVFPLAPSSKSTSGGTAALGCLVKDYFPEPVTVSWNSGALTSGVHTFPAVLQSSGLYSLSSVVTVPSSSLGTQTYICNVNHKPSNTKVDKKVEPKSCDKTHTCPPCPAPELLGGPSVFLFPPKPKDTLMISRTPEVTCVVVDVSHEDPEVKFNWYVDGVEVHNAKTKPREEQYNSTYRVVSVLTVLHQDWLNGKEYKCKVSNKALPAPIEKTISKAKGQPREPQVYTLPPSRDELTKNQVSLTCLVKGFYPSDIAVEWESNGQPENNYKTTPPVLDSDGSFFLYSKLTVDKSRWQQGNVFSCSVMHEALHNHYTQKSLSLSPGK

SEQ ID NO: 60 - protein, 217 aa, artificial
  reference antibody light chain
QSVLTQPPSVSGAPGQRVTISCTGSSSNIGSGYDVHWYQQLPGTAPKLLIYGNSKRPSGVPDRFSGSKSGTSASLAITGLQSEDEADYYCASWTDGLSLVVFGGGTKLTVLGQPKAAPSVTLFPPSSEELQANKATLVCLISDFYPGAVTVAWKADSSPVKAGVETTTPSKQSNNKYAASSYLSLTPEQWKSHRSYSCQVTHEGSTVEKTVAPTECS

SEQ ID NO: 61 - protein, 451 aa, artificial
  benchmark antibody heavy chain
EVQLVESGGGLVQPGRSLRLSCAASGFTFDDYAMHWVRQAPGKGLEWVSAITWNSGHIDYADSVEGRFTISRDNAKNSLYLQMNSLRAEDTAVYYCAKVSYLSTASSLDYWGQGTLVTVSSASTKGPSVFPLAPSSKSTSGGTAALGCLVKDYFPEPVTVSWNSGALTSGVHTFPAVLQSSGLYSLSSVVTVPSSSLGTQTYICNVNHKPSNTKVDKKVEPKSCDKTHTCPPCPAPELLGGPSVFLFPPKPKDTLMISRTPEVTCVVVDVSHEDPEVKFNWYVDGVEVHNAKTKPREEQYNSTYRVVSVLTVLHQDWLNGKEYKCKVSNKALPAPIEKTISKAKGQPREPQVYTLPPSREEMTKNQVSLTCLVKGFYPSDIAVEWESNGQPENNYKTTPPVLDSDGSFFLYSKLTVDKSRWQQGNVFSCSVMHEALHNHYTQKSLSLSPGK

SEQ ID NO: 62 - protein, 214 aa, artificial
  benchmark antibody light chain
DIQMTQSPSSLSASVGDRVTITCRASQGIRNYLAWYQQKPGKAPKLLIYAASTLQSGVPSRFSGSGSGTDFTLTISSLQPEDVATYYCQRYNRAPYTFGQGTKVEIKRTVAAPSVFIFPPSDEQLKSGTASVVCLLNNFYPREAKVQWKVDNALQSGNSQESVTEQDSKDSTYSLSSTLTLSKADYEKHKVYACEVTHQGLSSPVTKSFNRGEC

SEQ ID NO: 63 - protein, 619 aa, artificial
  fusion polypeptide
EVQLVESGGGLVQPGRSLRLSCAASGFTFDDYAMHWVRQAPGKGLEWVSAITWNSGHIDYADSVEGRFTISRDNAKNSLYLQMNSLRAEDTAVYYCAKVSYLSTASSLDYWGQGTLVTVSSASTKGPSVFPLAPSSKSTSGGTAALGCLVKDYFPEPVTVSWNSGALTSGVHTFPAVLQSSGLYSLSSVVTVPSSSLGTQTYICNVNHKPSNTKVDKKVEPKSCDKTHTCPPCPAPELLGGPSVFLFPPKPKDTLMISRTPEVTCVVVDVSHEDPEVKFNWYVDGVEVHNAKTKPREEQYNSTYRVVSVLTVLHQDWLNGKEYKCKVSNKALPAPIEKTISKAKGQPREPQVYTLPPSREEMTKNQVSLTCLVKGFYPSDIAVEWESNGQPENNYKTTPPVLDSDGSFFLYSKLTVDKSRWQQGNVFSCSVMHEALHNHYTQKSLSLSPGKGGGGSGGGGSGGGGSASDEEIQDVSGTWYLKAMTVDFWCSGIHEESVTPMTLTTLEGGNLEAKVTMDIEGFLQEFKAVLEKTDEPGKYTADGGKHVAYIIRSRVKDHYIFYSEGDCPGPVPGVWLVGRDPKNNLEALEDFEKAAGARGLSTESILIPRQSETSSPGSD

SEQ ID NO: 64 - protein, 644 aa, artificial
  fusion polypeptide
EVQLVESGGGLVQPGRSLRLSCAASGFTFDDYAMHWVRQAPGKGLEWVSAITWNSGHIDYADSVEGRFTISRDNAKNSLYLQMNSLRAEDTAVYYCAKVSYLSTASSLDYWGQGTLVTVSSASTKGPSVFPLAPSSKSTSGGTAALGCLVKDYFPEPVTVSWNSGALTSGVHTFPAVLQSSGLYSLSSVVTVPSSSLGTQTYICNVNHKPSNTKVDKKVEPKSCDKTHTCPPCPAPELLGGPSVFLFPPKPKDTLMISRTPEVTCVVVDVSHEDPEVKFNWYVDGVEVHNAKTKPREEQYNSTYRVVSVLTVLHQDWLNGKEYKCKVSNKALPAPIEKTISKAKGQPREPQVYTLPPSREEMTKNQVSLTCLVKGFYPSDIAVEWESNGQPENNYKTTPPVLDSDGSFFLYSKLTVDKSRWQQGNVFSCSVMHEALHNHYTQKSLSLSPGKGGGGSGGGGSGGGGSQDSTSDLIPAPPLSKVPLQQNFQDNQFHGKWYVVGEAGNLLLREDKDPRKMTATIYELKEDKSYDVTRVEFGAKTYKYQIGTFVPGSQPGEFTLGGIESMPGMTSFLVRVVSTNYNQHAIVFFKYVYQNREYFEITLYGRTKELTSELKENFIRFSKSLGLPENHIVFPVPIDQAIDG

SEQ ID NO: 65 - DNA, 1353 bp, artificial
  benchmark antibody heavy chain
gaagtgcagctggtcgaaagtggtggtggtctggtgcagcccggtagaagtctgcgtctgtcttgtgccgcatctggttttacattcgacgattacgcaatgcattgggtgagacaggcccccggcaagggactggagtgggtctccgctatcacctggaacagcgggcatattgactacgcagattccgtggaaggcaggttcacaatctctcgggacaacgccaagaatagtctgtatctgcagatgaattcactgagggccgaggataccgccgtgtactattgcgctaaagtctcttatctgtctaccgcatcatctctggattactggggtcagggaacactggtcactgtctcctctgctagcacaaagggccctagtgtgtttcctctggctccctcttccaaatccacttctggtggcactgctgctctgggatgcctggtgaaggattactttcctgaacctgtgactgtctcatggaactctggtgctctgacttctggtgtccacactttccctgctgtgctgcagtctagtggactgtactctctgtcatctgtggtcactgtgccctcttcatctctgggaacccagacctacatttgtaatgtgaaccacaaaccatccaacactaaagtggacaaaaaagtggaacccaaatcctgtgacaaaacccacacctgcccaccttgtcctgcccctgaactgctgggaggaccttctgtgtttctgttcccaccaaaaccaaaagataccctgatgatctctagaacccctgaggtgacatgtgtggtggtggatgtgtctcatgaggaccctgaggtcaaattcaactggtacgtggatggagtggaagtccacaatgccaaaaccaagcctagagaggaacagtacaattcaacctacagagtggtcagtgtgctgactgtgctgcatcaggattggctgaatggcaaggaatacaagtgtaaagtctcaaacaaggccctgcctgctccaattgagaaaacaatctcaaaggccaagggacagcctagggaaccccaggtctacaccctgccaccttcaagagaggaaatgaccaaaaaccaggtgtccctgacatgcctggtcaaaggcttctacccttctgacattgctgtggagtgggagtcaaatggacagcctgagaacaactacaaaacaaccccccctgtgctggattctgatggctctttctttctgtactccaaactgactgtggacaagtctagatggcagcaggggaatgtcttttcttgctctgtcatgcatgaggctctgcataaccactacactcagaaatccctgtctctgtctcctggcaaa

SEQ ID NO: 66 - DNA, 642 bp, artificial
  benchmark antibody light chain
gacatccagatgacccagagcccaagttccctgagcgcaagcgtcggagatcgtgtgactattacctgtagagcaagccagggcatcagaaactacctggcatggtatcagcagaagcccggtaaagcccctaagctgctgatctacgccgcttccactctgcagtctggcgtgccaagcaggttctctggcagtggatcagggaccgactttaccctgacaatttccagcctgcagcccgaggatgtcgctacatactattgccagcggtacaatcgggcaccttatacattcggtcaggggactaaagtggaaatcaagagaactgtcgcggcgccttctgtgttcattttccccccatctgatgaacagctgaaatctggcactgcttctgtggtctgtctgctgaacaacttctaccctagagaggccaaagtccagtggaaagtggacaatgctctgcagagtgggaattcccaggaatctgtcactgagcaggactctaaggatagcacatactccctgtcctctactctgacactgagcaaggctgattacgagaaacacaaagtgtacgcctgtgaagtcacacatcaggggctgtctagtcctgtgaccaaatccttcaataggggagagtgc

SEQ ID NO: 67 - DNA, 1857 bp, artificial
  fusion polypeptide
gaagtgcagctggtcgaaagtggtggtggtctggtgcagcccggtagaagtctgcgtctgtcttgtgccgcatctggttttacattcgacgattacgcaatgcattgggtgagacaggcccccggcaagggactggagtgggtctccgctatcacctggaacagcgggcatattgactacgcagattccgtggaaggcaggttcacaatctctcgggacaacgccaagaatagtctgtatctgcagatgaattcactgagggccgaggataccgccgtgtactattgcgctaaagtctcttatctgtctaccgcatcatctctggattactggggtcagggaacactggtcactgtctcctctgctagcacaaagggccctagtgtgtttcctctggctccctcttccaaatccacttctggtggcactgctgctctgggatgcctggtgaaggattactttcctgaacctgtgactgtctcatggaactctggtgctctgacttctggtgtccacactttccctgctgtgctgcagtctagtggactgtactctctgtcatctgtggtcactgtgccctcttcatctctgggaacccagacctacatttgtaatgtgaaccacaaaccatccaacactaaagtggacaaaaaagtggaacccaaatcctgtgacaaaacccacacctgcccaccttgtcctgcccctgaactgctgggaggaccttctgtgtttctgttcccaccaaaaccaaaagataccctgatgatctctagaacccctgaggtgacatgtgtggtggtggatgtgtctcatgaggaccctgaggtcaaattcaactggtacgtggatggagtggaagtccacaatgccaaaaccaagcctagagaggaacagtacaattcaacctacagagtggtcagtgtgctgactgtgctgcatcaggattggctgaatggcaaggaatacaagtgtaaagtctcaaacaaggccctgcctgctccaattgagaaaacaatctcaaaggccaagggacagcctagggaaccccaggtctacaccctgccaccttcaagagaggaaatgaccaaaaaccaggtgtccctgacatgcctggtcaaaggcttctacccttctgacattgctgtggagtgggagtcaaatggacagcctgagaacaactacaaaacaaccccccctgtgctggattctgatggctctttctttctgtactccaaactgactgtggacaagtctagatggcagcaggggaatgtcttttcttgctctgtcatgcatgaggctctgcataaccactacactcagaaatccctgtctctgtctcctggcaaaggcggcggaggatccggcggaggaggtagcggcggaggaggtagcgcatcagacgaggaaatccaggacgtgtcagggacctggtacctgaaagccatgaccgtggatttttggtgctccggcatccatgaggagtcagtcactcccatgaccctgacaaccctagaaggtgggaatctggaggccaaagtgacaatggatattgagggctttctccaggagttcaaagccgtcctcgagaagacagacgagcctggaaagtatactgctgatgggggaaaacacgtagcctatatcattcgatctcgggtgaaggatcattatatcttctattccgagggcgactgccccggccctgtgccaggtgtctggctagttgggagggaccccaagaacaatctcgaggctctggaggacttcgagaaggcagctggtgccaggggattgagcactgagtctatccttatcccacgccagagcgagacctcaagcccagggtccgac

SEQ ID NO: 68 - DNA, 1932 bp, artificial
  fusion polypeptide
gaagtgcagctggtcgaaagtggtggtggtctggtgcagcccggtagaagtctgcgtctgtcttgtgccgcatctggttttacattcgacgattacgcaatgcattgggtgagacaggcccccggcaagggactggagtgggtctccgctatcacctggaacagcgggcatattgactacgcagattccgtggaaggcaggttcacaatctctcgggacaacgccaagaatagtctgtatctgcagatgaattcactgagggccgaggataccgccgtgtactattgcgctaaagtctcttatctgtctaccgcatcatctctggattactggggtcagggaacactggtcactgtctcctctgctagcacaaagggccctagtgtgtttcctctggctccctcttccaaatccacttctggtggcactgctgctctgggatgcctggtgaaggattactttcctgaacctgtgactgtctcatggaactctggtgctctgacttctggtgtccacactttccctgctgtgctgcagtctagtggactgtactctctgtcatctgtggtcactgtgccctcttcatctctgggaacccagacctacatttgtaatgtgaaccacaaaccatccaacactaaagtggacaaaaaagtggaacccaaatcctgtgacaaaacccacacctgcccaccttgtcctgcccctgaactgctgggaggaccttctgtgtttctgttcccaccaaaaccaaaagataccctgatgatctctagaacccctgaggtgacatgtgtggtggtggatgtgtctcatgaggaccctgaggtcaaattcaactggtacgtggatggagtggaagtccacaatgccaaaaccaagcctagagaggaacagtacaattcaacctacagagtggtcagtgtgctgactgtgctgcatcaggattggctgaatggcaaggaatacaagtgtaaagtctcaaacaaggccctgcctgctccaattgagaaaacaatctcaaaggccaagggacagcctagggaaccccaggtctacaccctgccaccttcaagagaggaaatgaccaaaaaccaggtgtccctgacatgcctggtcaaaggcttctacccttctgacattgctgtggagtgggagtcaaatggacagcctgagaacaactacaaaacaaccccccctgtgctggattctgatggctctttctttctgtactccaaactgactgtggacaagtctagatggcagcaggggaatgtcttttcttgctctgtcatgcatgaggctctgcataaccactacactcagaaatccctgtctctgtctcctggcaaaggcggcggaggatccgggggtgggggaagcggcggaggaggtagccaggattcaaccagcgatctgattccagcaccgccactgtcgaaagtgccactgcaacaaaactttcaagataaccagtttcacggcaagtggtatgtggtcggggaggccggtaacctgctgctgagggaagacaaagatccacggaaaatgaccgccaccatctacgagctgaaagaggataagtcctacgacgtgactcgggtggagttcggcgcaaaaacctacaagtaccagatcggcaccttcgtgcccggctctcagcctggcgagtttaccctgggcggcatcgaatctatgcccggcatgaccagctttctcgtgcgggtggtgtccaccaactacaaccagcacgccatcgtgttcttcaaatacgtgtaccagaaccgcgagtacttcgagatcaccctgtacggccggaccaaagagctgacctccgaactgaaagagaacttcatccggttctccaagtccctgggcctgcccgagaaccacatcgtgttccccgtgcctatcgaccaggccatcgacggc